European Patent Specification EP 3 816 277 B1, published February 19, 2025. Title: Pancreatic Organoid Derived from Mutant Mouse and Use thereof and Standardized Method for Identifying Drug Efficacy. Applicant: Seoul National University R&DB Foundation. The sequence listing filed with the application follows.

SEQUENCE LISTING (11 sequences)

SEQ ID NO: 1 - DNA, 23 bp, Artificial Sequence
  Brca2-11F primer
ctcatcatttgttgcctcacttc

SEQ ID NO: 2 - DNA, 21 bp, Artificial Sequence
  Brca2-11R primer
tgttggatacaaggcatgtac

SEQ ID NO: 3 - DNA, 20 bp, Artificial Sequence
  mTR-WT primer
gcactccttacaagggacga

SEQ ID NO: 4 - DNA, 20 bp, Artificial Sequence
  mTR-common primer
cttcaatttccttggcttcg

SEQ ID NO: 5 - DNA, 22 bp, Artificial Sequence
  mTR-mutant primer
atttgtcacgtcctgcacgacg

SEQ ID NO: 6 - DNA, 20 bp, Artificial Sequence
  CRE-3F primer
cggcatggtgcaagttgaat

SEQ ID NO: 7 - DNA, 20 bp, Artificial Sequence
  CRE-3R primer
cggtgctaaccagcgttttc

SEQ ID NO: 8 - DNA, 24 bp, Artificial Sequence
  CRE-internal-F primer
ctaggccacagaattgaaagatct

SEQ ID NO: 9 - DNA, 25 bp, Artificial Sequence
  CRE-internal-R primer
gtaggtggaaattctagcatcatcc

SEQ ID NO: 10 - DNA, 20 bp, Artificial Sequence
  BubR1K243R/+ F primer
gaggtaaaggcaggggaatc

SEQ ID NO: 11 - DNA, 20 bp, Artificial Sequence
  BubR1K243R/+ R primer
gagaaagcgggggtcattat